European Patent Application EP 4 810 626 A1, published September 23, 2026. Title: 一种寡核苷酸集合以及多重扩增子建库方法. Applicant: 南京诺唯赞生物科技股份有限公司. Application CN. The sequence listing filed with the application follows.

SEQUENCE LISTING (28 sequences)

SEQ ID NO: 1 - DNA, 60 bp, synthetic construct
  source 1..60: mol_type = other DNA
tgcttatcaatggatttatatttgtgactgtctcttatacacatctgacgctgccgacga

SEQ ID NO: 2 - DNA, 64 bp, synthetic construct
  source 1..64: mol_type = other DNA
cccattaggatatttcaaaggtatataaagctgtctcttatacacatctccgagcccacgagac

SEQ ID NO: 3 - DNA, 60 bp, synthetic construct; identical to SEQ ID NO: 1
  source 1..60: mol_type = other DNA
  modified_base 8: mod_base = OTHER; note = cytidine in RNA
  modified_base 19: mod_base = OTHER; note = uracil
  modified_base 27: mod_base = OTHER; note = adenine in RNA

SEQ ID NO: 4 - DNA, 64 bp, synthetic construct; identical to SEQ ID NO: 2
  source 1..64: mol_type = other DNA
  modified_base 8: mod_base = OTHER; note = guanine in RNA
  modified_base 22: mod_base = OTHER; note = uracil
  modified_base 30: mod_base = OTHER; note = guanine in RNA

SEQ ID NO: 5 - DNA, 27 bp, synthetic construct
  source 1..27: mol_type = other DNA
tcacaaatataaatccattgataagca

SEQ ID NO: 6 - DNA, 30 bp, synthetic construct
  source 1..30: mol_type = other DNA
ctttatatacctttgaaatatcctaatggg

SEQ ID NO: 7 - DNA, 60 bp, synthetic construct
  source 1..60: mol_type = other DNA
tcgtcggcagcgtcagatgtgtataagagacagtcacaaatataaatccattgataagca

SEQ ID NO: 8 - DNA, 64 bp, synthetic construct
  source 1..64: mol_type = other DNA
gtctcgtgggctcggagatgtgtataagagacagctttatatacctttgaaatatcctaatggg

SEQ ID NO: 9 - DNA, 22 bp, synthetic construct
  source 1..22: mol_type = other DNA
  modified_base 9: mod_base = OTHER; note = guanine in RNA
  modified_base 17: mod_base = OTHER; note = guanine in RNA
tcttgagtgagacgctgccgac

SEQ ID NO: 10 - DNA, 20 bp, synthetic construct
  source 1..20: mol_type = other DNA
  modified_base 8: mod_base = OTHER; note = adenine in RNA
  modified_base 15: mod_base = OTHER; note = guanine in RNA
gctgttgatgccgagcccac

SEQ ID NO: 11 - DNA, 56 bp, synthetic construct
  source 1..56: mol_type = other DNA
tcactcaagaagatgtgtataagagacagtcacaaatataaatccattgataagca

SEQ ID NO: 12 - DNA, 59 bp, synthetic construct
  source 1..59: mol_type = other DNA
catcaacagcagatgtgtataagagacagctttatatacctttgaaatatcctaatggg

SEQ ID NO: 13 - DNA, 24 bp, synthetic construct
  source 1..24: mol_type = other DNA
tcttatacacatctgacgctgccg

SEQ ID NO: 14 - DNA, 23 bp, synthetic construct
  source 1..23: mol_type = other DNA
gacaggatgcagatcggaagagc

SEQ ID NO: 15 - DNA, 23 bp, synthetic construct
  source 1..23: mol_type = other DNA
ctagggacttagatcggaagagc

SEQ ID NO: 16 - DNA, 24 bp, synthetic construct
  source 1..24: mol_type = other DNA
tcttatacacatctccgagcccac

SEQ ID NO: 17 - DNA, 46 bp, synthetic construct
  source 1..46: mol_type = other DNA
agatgtgtataagagacagtcacaaatataaatccattgataagca

SEQ ID NO: 18 - DNA, 40 bp, synthetic construct
  source 1..40: mol_type = other DNA
gcatcctgtcctttatatacctttgaaatatcctaatggg

SEQ ID NO: 19 - DNA, 37 bp, synthetic construct
  source 1..37: mol_type = other DNA
aagtccctagtcacaaatataaatccattgataagca

SEQ ID NO: 20 - DNA, 49 bp, synthetic construct
  source 1..49: mol_type = other DNA
agatgtgtataagagacagctttatatacctttgaaatatcctaatggg

SEQ ID NO: 21 - DNA, 22 bp, synthetic construct
  source 1..22: mol_type = other DNA
aatgatacggcgaccaccgaga

SEQ ID NO: 22 - DNA, 22 bp, synthetic construct
  source 1..22: mol_type = other DNA
caagcagaagacggcatacgag

SEQ ID NO: 23 - DNA, 30 bp, synthetic construct
  source 1..30: mol_type = other DNA
gcatcctgtccgagacgtgtcaaatggctg

SEQ ID NO: 24 - DNA, 30 bp, synthetic construct
  source 1..30: mol_type = other DNA
gcatcctgtctggtacgacgcaaatcggta

SEQ ID NO: 25 - DNA, 53 bp, synthetic construct
  source 1..53: mol_type = other DNA
tcgtcggcagcgtcagatgtgtataagagacagcgagacgtgtcaaatggctg

SEQ ID NO: 26 - DNA, 53 bp, synthetic construct
  source 1..53: mol_type = other DNA
tcgtcggcagcgtcagatgtgtataagagacagtggtacgacgcaaatcggta

SEQ ID NO: 27 - DNA, 53 bp, synthetic construct
  source 1..53: mol_type = other DNA
  modified_base 7: mod_base = OTHER; note = uracil
  modified_base 13: mod_base = OTHER; note = adenine in RNA
  modified_base 20: mod_base = OTHER; note = guanine in RNA
cagccatttgacacgtctcgctgtctcttatacacatctgacgctgccgacga

SEQ ID NO: 28 - DNA, 53 bp, synthetic construct
  source 1..53: mol_type = other DNA
  modified_base 7: mod_base = OTHER; note = Uracil
  modified_base 13: mod_base = OTHER; note = Uracil
  modified_base 20: mod_base = OTHER; note = adenine in RNA
taccgatttgcgtcgtaccactgtctcttatacacatctgacgctgccgacga